European Patent Specification EP 3 947 351 B1, published March 11, 2026. Title: SMALL MOLECULE PARG INHIBITORS AND METHODS OF USE THEREOF. Applicant: BOARD OF REGENTS, THE UNIVERSITY OF TEXAS SYSTEM BOARD OF TRUSTEES OF THE UNIVERSITY OF ARKANSAS WASHINGTON UNIVERSITY. Application Unknown. The sequence listing filed with the application follows.

SEQUENCE LISTING (9 sequences)

SEQ ID NO: 1 - DNA, 57 bp, Artificial sequence
  Synthetic plasmid
gatccggaaacggtactctactaattcaagagattagtagagtaccgtttccttttt

SEQ ID NO: 2 - DNA, 21 bp, Artificial sequence
  Synthetic plasmid
ggaaacgguacucuacuaatt

SEQ ID NO: 3 - DNA, 21 bp, Artificial sequence
  Synthetic plasmid
uuaguagaguaccguuucctt

SEQ ID NO: 4 - DNA, 57 bp, Artificial sequence
  Synthetic plasmid
gatccgaaggatgctattctgaaattcaagagatttcagaatagcatccttcttttt

SEQ ID NO: 5 - DNA, 21 bp, Artificial sequence
  Synthetic plasmid
gaaggaugcuauucugaaatt

SEQ ID NO: 6 - DNA, 21 bp, Artificial sequence
  Synthetic plasmid
uuucagaauagcauccuuctt

SEQ ID NO: 7 - DNA, 57 bp, Artificial sequence
  Synthetic plasmid
gatccggaaaccggagaaacttaattcaagagattaagtttctccggtttccttttt

SEQ ID NO: 8 - DNA, 21 bp, Artificial sequence
  Synthetic plasmid
ggaaaccggagaaacuuaatt

SEQ ID NO: 9 - DNA, 21 bp, Artificial sequence
  Synthetic plasmid
uuaaguuucuccgguuucctt